European Patent Specification EP 4 031 683 B1, published September 2, 2026. Title: STRUCTURE AND TEMPERATURE-DEPENDENT FLAP ENDONUCLEASE SUBSTRATES. Applicant: EXACT SCIENCES DEVELOPMENT COMPANY, LLC. The sequence listing filed with the application follows.

SEQUENCE LISTING (17 sequences)

SEQ ID NO: 1 - DNA, 85 bp, ArtIficial Sequence
  Synthetic
caccaacctcataaccttatcacacaaaccaatattaatacctacacccacaacactatcttaaacacctaatcaaaaaaacaaa

SEQ ID NO: 2 - DNA, 30 bp, Artificial Sequence
  Synthetic
gtgtttgtttttttgattaggtgtttaaga

SEQ ID NO: 3 - DNA, 26 bp, Artificial Sequence
  Synthetic
ctttacaccaacctcataaccttatc

SEQ ID NO: 4 - DNA, 21 bp, Artificial Sequence
  Synthetic
gacgcggagatagtgttgtgg

SEQ ID NO: 5 - DNA, 10 bp, Artificial Sequence
  Synthetic
gacgcggaga

SEQ ID NO: 6 - DNA, 32 bp, Artificial Sequence
  Synthetic
tctagccggttttccggctgagactccgcgtc

SEQ ID NO: 7 - DNA, 47 bp, Artificial Sequence
  Synthetic
cagttttctgttcttagccggttttccggctaagacgtccgtggcct

SEQ ID NO: 8 - DNA, 49 bp, Artificial Sequence
  Synthetic
caacttttgttgttcttagccggttttccggctaagacgtccgtggcct

SEQ ID NO: 9 - DNA, 48 bp, Artificial Sequence
  Synthetic
cgcttttctcgttcttagccggttttccggctaagacgtccgtggcct

SEQ ID NO: 10 - DNA, 41 bp, Artificial Sequence
  Synthetic
tcttagccggttttccggctgagactccgcttttgcggagg

SEQ ID NO: 11 - DNA, 53 bp, Artificial Sequence
  Synthetic
tcttagccggttttccggctgagacgtccgtggcctttttaggccacggacgg

SEQ ID NO: 12 - DNA, 68 bp, Artificial Sequence
  Synthetic
tccttattacttttgtaataaggattcttcagccggttttccggctgaagactccgcttttgcggagg

SEQ ID NO: 13 - DNA, 64 bp, Artificial Sequence
  Synthetic
tccttattacgtaataaggattcttcagccggttttccggctgaagactccgcttttgcggagg

SEQ ID NO: 14 - DNA, 64 bp, Artificial Sequence; identical to SEQ ID NO: 13
  Synthetic

SEQ ID NO: 15 - DNA, 54 bp, Artificial Sequence
  Synthetic
gtcttttgacttcttcagccggttttccggctgaagacgccgcttttgcggcgg

SEQ ID NO: 16 - DNA, 56 bp, Artificial Sequence
  Synthetic
gtcatttttgacttcttcagccggttttccggctgaagacgccgcttttgcggcgg

SEQ ID NO: 17 - DNA, 54 bp, Artificial Sequence
  Synthetic
gtcacgtgacttcttcagccggttttccggctgaagacgccgcttttgcggcgg